European Patent Application EP 4 768 576 A1, published July 1, 2026. Title: 嘌呤核苷磷酸化酶突变体及2'-氟代核苷的制备方法. Applicant: 吉林凯莱英制药有限公司. The sequence listing filed with the application follows.

SEQUENCE LISTING (6 sequences)

SEQ ID NO: 1 - protein, 423 aa, Thermus thermophilus
MNPVAFIREKREGKKHRREDLEAFLLGYLHDEVPDYQVSAWLMAAFLRGLDPEETLWLTETMARSGKVLDLSGLPHPVDQHSSGGVGDKVSLVVGPILAASGCTFAKMSGRTLAHTGGNIDKLESVPGWRGEMTEAEFLERARRVGLVIAAQSPDLTPLDGKLYALRDVTATTESVPLIASSIMSKKLAVGARSIVLDVKVGRGAFMKTLEEARLLAKTMVAIGQGDGRRVRALLTSMEAPLGRAVGNAIEVREAIEALKGEGPGDLLEVALALAEEALRREGLDPALARKALEGGAALEKFRAFLEAQGGDPRAVEDFSLLPLAEEHPLRAEREGVVREVDAYKVGLAVLALGGGRKRKGEPIDHGVGVYLLKKPGDRVERGEALALVYHRRRGLEEALGHLREAYALGEEAHPAPLVLEAI

SEQ ID NO: 2 - DNA, 1272 bp, synthetic construct
  source 1..1272: mol_type = other DNA; note; note (original language) = 编码嘧啶核苷磷酸化酶的DNA序列
atgaacccggtggcgtttattcgcgaaaaacgcgaaggcaagaaacatcgccgcgaggatctggaagcgtttctgctgggctatctgcacgatgaagtgccggattatcaggtgagcgcgtggctgatggcggcgtttttacgcggcttagatccggaagaaaccctgtggctgaccgaaacgatggcccgcagcggtaaagtgctggatctgagcggtctgccgcatccggttgatcagcatagcagcggcggcgtgggcgataaagtgagcttagtggtgggcccgattctggcggcgagcggttgtacctttgcgaaaatgtcgggccgcaccctggcgcataccggtggtaacattgataaactggaaagcgtgccgggctggcgcggcgaaatgaccgaagcagaatttctggaacgcgcccgtcgcgttggtctggttattgcggcgcaaagcccggatttaacgccgttagatggcaaactgtatgcgctgcgcgatgtgaccgcgaccactgaatcagttccgctgattgcgagcagcattatgagcaagaaactggcggtgggcgcccgtagcattgtgttagatgttaaagtgggccgcggcgcgtttatgaaaaccctggaagaagcgcgtctgctggcgaaaacgatggtggcgattggccagggcgatggccgtcgtgttcgtgcgttattaaccagcatggaagcgcctctgggtcgtgcggttggcaatgcgattgaagtgcgtgaagcgattgaagcgctgaaaggcgaaggcccgggcgatttattagaagtggcgctggcgttagcggaagaagcgctgcgtcgtgaaggcttagatccggcgctggcgcgtaaagcgttagaaggtggcgcggcgctggaaaaatttcgcgcgtttctggaagcgcagggcggcgatccgcgtgcagttgaagattttagcctgctgccgctggcggaagaacatccgttacgtgcggaacgcgaaggcgtggttcgcgaagttgatgcgtataaagtgggcctggcggtgctggcgttaggcggtggtcgtaaacgtaaaggtgaaccgattgatcatggcgtgggcgtgtatctgctgaagaaaccgggcgatcgcgtggaacgcggcgaagcgttagcgttagtgtatcatcgccgccgcggcttagaagaagcgctgggtcatttacgcgaagcgtatgcgctgggcgaagaagcgcatccggcgcctctggttttagaagcgatttaa

SEQ ID NO: 3 - protein, 234 aa, Geobacillus stearothermophilus
MSVHIGAKEHEIADKILLPGDPLRAKYIAETFLEGATCYNQVRGMLGFTGTYKGHRISVQGTGMGVPSISIYITELMQSYNVQTLIRVGTCGAIQKDVKVRDVILAMTSSTDSQMNRMTFGGIDYAPTANFDLLKTAYEIGKEKGLQLKVGSVFTADMFYNENAQFEKLARYGVLAVEMETTALYTLAAKFGRKALSVLTVSDHILTGEETTAEERQTTFNEMIEVALETAIRQ

SEQ ID NO: 4 - DNA, 705 bp, synthetic construct
  source 1..705: mol_type = other DNA; note; note (original language) = 编码嘌呤核苷磷酸化酶的DNA序列
atgagcgtgcatattggcgcgaaagaacatgaaattgcggataaaattctgctgccgggcgatccgttacgcgcgaaatatattgcggaaacctttctggaaggcgcgacctgctataaccaggtgcgcggcatgctgggctttaccggcacctataaaggccatcgcattagcgtgcagggcaccggcatgggcgttcctagcatttcaatttatattaccgaactgatgcagagctataacgtgcagaccctgattcgcgtgggcacctgcggtgcgattcaaaaagatgtgaaagtgcgcgatgtgattctggcgatgaccagcagcaccgatagccagatgaaccgcatgacctttggcggcattgattatgcgccgaccgcgaactttgatctgctgaaaaccgcgtatgaaattggcaaagaaaaaggcctgcagctgaaagtgggcagcgtgtttaccgcggatatgttttataacgaaaacgcgcagtttgagaaactggcccgctatggcgtgctggcggttgaaatggaaaccaccgcgctgtataccctggcggcgaaatttggccgcaaagcgctgagcgtgctgaccgtgagcgatcatattctgaccggcgaagaaaccaccgcggaagaacgccagaccacctttaacgaaatgattgaagtggcgctggaaaccgcgattcgccagtaa

SEQ ID NO: 5 - protein, 234 aa, synthetic construct
  source 1..234: note; note (original language) = GsPNP突变体
MSVHIGAKEHEIADKILLMGDPLRAKYIAETFLEGATCYNTVRGMLGFTGTYKGHRISVQGTGMGVPSMSIYATELMQSYNVQTLIRVGTCGAIQKDVKVRDVILAMTSSTDNQMNRMTFGGIDFSPCADFDLLKTAYEIGKELGLQPKVGSVFTADMFYNENAQFEKLARYGVKAVEMETTALYTLAAKFGRKALSVLTVSDHVLTGEETTAEERQTTFNEMIEVALETAIRQ

SEQ ID NO: 6 - DNA, 705 bp, synthetic construct
  source 1..705: mol_type = other DNA; note; note (original language) = 编码GsPNP突变体的DNA序列
atgagcgtgcatattggcgcgaaagaacatgaaattgcggataaaattctgctgatgggcgatccgttacgcgcgaaatatattgcggaaacctttctggaaggcgcgacctgctataacaccgtgcgcggcatgctgggctttaccggcacctataaaggccatcgcattagcgtgcagggcaccggcatgggcgttcctagcatgtcaatttatgctaccgaactgatgcagagctataacgtgcagaccctgattcgcgtgggcacctgcggtgcgattcaaaaagatgtgaaagtgcgcgatgtgattctggcgatgaccagcagcaccgataaccagatgaaccgcatgacctttggcggcattgattttagtccgtgcgcggactttgatctgctgaaaaccgcgtatgaaattggcaaagaactgggcctgcagccgaaagtgggcagcgtgtttaccgcggatatgttttataacgaaaacgcgcagtttgagaaactggcccgctatggcgtgaaggcggttgaaatggaaaccaccgcgctgtataccctggcggcgaaatttggccgcaaagcgctgagcgtgctgaccgtgagcgatcatgttctgaccggcgaagaaaccaccgcggaagaacgccagaccacctttaacgaaatgattgaagtggcgctggaaaccgcgattcgccagtaa